European Patent Specification EP 4 082 538 B1, published February 14, 2024. Title: METHODS AND COMPOSITIONS FOR TREATMENT OF MUSCLE WASTING, MUSCLE WEAKNESS AND/OR CACHEXIA. Applicant: Baylor College of Medicine. The sequence listing filed with the application follows.

SEQUENCE LISTING (25 sequences)

SEQ ID NO: 1 - DNA, 22 bp, Artificial Sequence
  Synthetic Primer
tctacatcttactcctgttgat

SEQ ID NO: 2 - DNA, 23 bp, Artificial Sequence
  Synthetic Primer
caaatgctgctttattcttacaa

SEQ ID NO: 3 - DNA, 18 bp, Artificial Sequence
  Synthetic Primer
caacctgaatccaactta

SEQ ID NO: 4 - DNA, 18 bp, Artificial Sequence
  Synthetic Primer
tgttaccttgacctctaa

SEQ ID NO: 5 - DNA, 18 bp, Artificial Sequence
  Synthetic Primer
ttacaatctgcctcaatc

SEQ ID NO: 6 - DNA, 18 bp, Artificial Sequence
  Synthetic Primer
atctcctaatagcctcaa

SEQ ID NO: 7 - DNA, 21 bp, Artificial Sequence
  Synthetic Primer
ctctggtaaagtggatattgt

SEQ ID NO: 8 - DNA, 20 bp, Artificial Sequence
  Synthetic Primer
ggtggaatcatattggaaca

SEQ ID NO: 9 - DNA, 18 bp, Artificial Sequence
  Synthetic Primer
caacctcttctggctcaa

SEQ ID NO: 10 - DNA, 18 bp, Artificial Sequence
  Synthetic Primer
tggtggtcttgttgctta

SEQ ID NO: 11 - DNA, 22 bp, Artificial Sequence
  Synthetic Primer
ctccagggtctaaatacatagc

SEQ ID NO: 12 - DNA, 18 bp, Artificial Sequence
  Synthetic Primer
ctcacagcagtccacaag

SEQ ID NO: 13 - DNA, 21 bp, Artificial Sequence
  Synthetic Primer
cacagcaagtttcccgccgcc

SEQ ID NO: 14 - DNA, 21 bp, Artificial Sequence
  Synthetic Primer
gtgcaccagcttgagtacaca

SEQ ID NO: 15 - DNA, 19 bp, Artificial Sequence
  Synthetic Primer
ctccagaatagaagccata

SEQ ID NO: 16 - DNA, 19 bp, Artificial Sequence
  Synthetic Primer
gcagaagttgtcttatagc

SEQ ID NO: 17 - DNA, 24 bp, Artificial Sequence
  Synthetic Primer
gaggcagattcgcaagcgtttgat

SEQ ID NO: 18 - DNA, 24 bp, Artificial Sequence
  Synthetic Primer
tccaggagagaatgtggcagtgtt

SEQ ID NO: 19 - DNA, 24 bp, Artificial Sequence
  Synthetic Primer
agtgtccatgtctggaggtcgttt

SEQ ID NO: 20 - DNA, 24 bp, Artificial Sequence
  Synthetic Primer
actggagcactcctgcttgtagat

SEQ ID NO: 21 - DNA, 20 bp, Artificial Sequence
  Synthetic Primer
accaccatggagaaggccgg

SEQ ID NO: 22 - DNA, 20 bp, Artificial Sequence
  Synthetic Primer
ctcagtgtagcccaagatgc

SEQ ID NO: 23 - protein, 4 aa, Artificial Sequence
  Synthetic Peptide
  MISC_FEATURE (4)..(4): 7-amino-4-methylcoumarin (AMC) tag
LLVY

SEQ ID NO: 24 - protein, 101 aa, Artificial Sequence
  Synthetic Peptide
NEGYIMGFISKERERAILSTKPPGTFLLRFSESSKEGGVTFTWVEKDISGSTQIQSVEPYTKQQLNNMSFAEIIMGYKIMDATNILVSPLVYLYPDIPKEE

SEQ ID NO: 25 - protein, 102 aa, Artificial Sequence
  Synthetic Peptide
NDGCIMGFISKERERALLKDQQPGTFLLRFSESSREGAITFTWVERSQNGGEPDGHAVEPYTKKELSAVTFPDIIRNYKVMAAENIPENPLKYLYPNIDKDH